European Patent Specification EP 3 778 629 B1, published April 26, 2023. Title: APPLICATION OF RYR2 PROTEIN OR RECOMBINANT RYR2 PROTEIN IN PREPARING ANTI-HEART FAILURE MEDICAMENT. Applicant: PHARCHOICE THERAPEUTICS INC. The sequence listing filed with the application follows.

SEQUENCE LISTING (30 sequences)

SEQ ID NO: 1 - protein, 189 aa, Artificial Sequence
  The sequence is synthetized.
VSSMRPNIFLGVSEGSAQYKKWYYELMVDHTEPFVTAEATHLRVGWASTEGYSPYPGGGEEWGGNGVGDDLFSYGFDGLHLWSGCIARTVSSPNQHLLRTDDVISCCLDLSAPSISFRINGQPVQGMFENFNIDGLFFPVVSFSAGIKVRFLLGGRHGEFKFLPPPGYAPCYEAVLPKEKLKVEHSREY

SEQ ID NO: 2 - DNA, 567 bp, Artificial Sequence
  The sequence is synthetized.
gtgagcagcatgagacccaacatcttcctgggcgtgagcgagggcagcgcccagtacaagaagtggtactacgagctgatggtggaccacaccgagcccttcgtgaccgccgaggccacccacctgagagtgggctgggccagcaccgagggctacagcccctaccccggcggcggcgaggagtggggcggcaacggcgtgggcgacgacctgttcagctacggcttcgacggcctgcacctgtggagcggctgcatcgccagaaccgtgagcagccccaaccagcacctgctgagaaccgacgacgtgatcagctgctgcctggacctgagcgcccccagcatcagcttcagaatcaacggccagcccgtgcagggcatgttcgagaacttcaacatcgacggcctgttcttccccgtggtgagcttcagcgccggcatcaaggtgagattcctgctgggcggcagacacggcgagttcaagttcctgcccccccccggctacgccccctgctacgaggccgtgctgcccaaggagaagctgaaggtggagcacagcagagagtac

SEQ ID NO: 3 - protein, 205 aa, Artificial Sequence
  The sequence is synthetized.
FTPIPVDTSQIVLPPHLERIREKLAENIHELWVMNKIELGWQYGPVRDDNKRQHPCLVEFSKLPEQERNYNLQMSLETLKTLLALGCHVGISDEHAEDKVKKMKLPKNYQLTSGYKPAPMDLSFIKLTPSQEAMVDKLAENAHNVWARDRIRQGWTYGIQQDVKNRRNPRLVPYTLLDDRTKKSNKDSLREAVRTLLGYGYNLEA

SEQ ID NO: 4 - DNA, 615 bp, Artificial Sequence
  The sequence is synthetized.
ttcacccccatccccgtggacaccagccagatcgtgctgcccccccacctggagagaatcagagagaagctggccgagaacatccacgagctgtgggtgatgaacaagatcgagctgggctggcagtacggccccgtgagagacgacaacaagagacagcacccctgcctggtggagttcagcaagctgcccgagcaggagagaaactacaacctgcagatgagcctggagaccctgaagaccctgctggccctgggctgccacgtgggcatcagcgacgagcacgccgaggacaaggtgaagaagatgaagctgcccaagaactaccagctgaccagcggctacaagcccgcccccatggacctgagcttcatcaagctgacccccagccaggaggccatggtggacaagctggccgagaacgcccacaacgtgtgggccagagacagaatcagacagggctggacctacggcatccagcaggacgtgaagaacagaagaaaccccagactggtgccctacaccctgctggacgacagaaccaagaagagcaacaaggacagcctgagagaggccgtgagaaccctgctgggctacggctacaacctggaggcc

SEQ ID NO: 5 - protein, 134 aa, Artificial Sequence
  The sequence is synthetized.
RFRIFRAEKTYAVKAGRWYFEFETVTAGDMRVGWSRPGCQPDQELGSDERAFAFDGFKAQRWHQGNEHYGRSWQAGDVVGCMVDMNEHTMMFTLNGEILLDDSGSELAFKDFDVGDGFIPVCSLGVAQVGRMNF

SEQ ID NO: 6 - DNA, 402 bp, Artificial Sequence
  The sequence is synthetized.
agattcagaatcttcagagccgagaagacctacgccgtgaaggccggcagatggtacttcgagttcgagaccgtgaccgccggcgacatgagagtgggctggagcagacccggctgccagcccgaccaggagctgggcagcgacgagagagccttcgccttcgacggcttcaaggcccagagatggcaccagggcaacgagcactacggcagaagctggcaggccggcgacgtggtgggctgcatggtggacatgaacgagcacaccatgatgttcaccctgaacggcgagatcctgctggacgacagcggcagcgagctggccttcaaggacttcgacgtgggcgacggcttcatccccgtgtgcagcctgggcgtggcccaggtgggcagaatgaacttc

SEQ ID NO: 7 - protein, 398 aa, Artificial Sequence
  The sequence is synthetized.
NRDITMWLSKRLPQFLQVPSNHEHIEVTRIDGTIDSSPCLKVTQKSFGSQNSNTDIMFYRLSMPIECAEVFSKTVAGGLPGAGLFGPKNDLEDYDADSDFEVLMKTAHGHLVPDRVDKDKEATKPEFNNHKDYAQEKPSRLKQRFLLRRTKPDYSTSHSARLTEDVLADDRDDYDFLMQTSTYYYSVRIFPGQEPANVWVGWITSDFHQYDTGFDLDRVRTVTVTLGDEKGKVHESIKRSNCYMVCAGESMSPGQGRNNNGLEIGCVVDAASGLLTFIANGKELSTYYQVEPSTKLFPAVFAQATSPNVFQFELGRIKNVMPLSAGLFKSEHKNPVPQCPPRLHVQFLSHVLWSRMPNQFLKVDVSRISERQGWLVQCLDPLQFMSLHIPEENRSVDI

SEQ ID NO: 8 - DNA, 1194 bp, Artificial Sequence
  The sequence is synthetized.
aacagagacatcaccatgtggctgagcaagagactgccccagttcctgcaggtgcccagcaaccacgagcacatcgaggtgaccagaatcgacggcaccatcgacagcagcccctgcctgaaggtgacccagaagagcttcggcagccagaacagcaacaccgacatcatgttctacagactgagcatgcccatcgagtgcgccgaggtgttcagcaagaccgtggccggcggcctgcccggcgccggcctgttcggccccaagaacgacctggaggactacgacgccgacagcgacttcgaggtgctgatgaagaccgcccacggccacctggtgcccgacagagtggacaaggacaaggaggccaccaagcccgagttcaacaaccacaaggactacgcccaggagaagcccagcagactgaagcagagattcctgctgagaagaaccaagcccgactacagcaccagccacagcgccagactgaccgaggacgtgctggccgacgacagagacgactacgacttcctgatgcagaccagcacctactactacagcgtgagaatcttccccggccaggagcccgccaacgtgtgggtgggctggatcaccagcgacttccaccagtacgacaccggcttcgacctggacagagtgagaaccgtgaccgtgaccctgggcgacgagaagggcaaggtgcacgagagcatcaagagaagcaactgctacatggtgtgcgccggcgagagcatgagccccggccagggcagaaacaacaacggcctggagatcggctgcgtggtggacgccgccagcggcctgctgaccttcatcgccaacggcaaggagctgagcacctactaccaggtggagcccagcaccaagctgttccccgccgtgttcgcccaggccaccagccccaacgtgttccagttcgagctgggcagaatcaagaacgtgatgcccctgagcgccggcctgttcaagagcgagcacaagaaccccgtgccccagtgcccccccagactgcacgtgcagttcctgagccacgtgctgtggagcagaatgcccaaccagttcctgaaggtggacgtgagcagaatcagcgagagacagggctggctggtgcagtgcctggaccccctgcagttcatgagcctgcacatccccgaggagaacagaagcgtggacatc

SEQ ID NO: 9 - protein, 458 aa, Artificial Sequence
  The sequence is synthetized.
KFHYHTLRLYSAVCALGNHRVAHALCSHVDEPQLLYAIENKYMPGLLRAGYYDLLIDIHLSSYATARLMMNNEYIVPMTEETKSITLFPDENKKHGLPGIGLSTSLRPRMQFSSPSFVSISNECYQYSPEFPLDILKSKTIQMLTEAVKEGSLHARDPVGGTTEFLFVPLIKLFYTLLIMGIFHNEDLKHILQLIEPSVFKEAATPEEESDTLEKELSVDDAKLQGAGEEEAKGGKRPKEGLLQMKLPEPVKLQMCLLLQYLCDCQVRHRIEAIVAFSDDFVAKLQDNQRFRYNEVMQALNMSAALTARKTKEFRSPPQEQINMLLNFKDDKSECPCPEEIRDQLLDFHEDLMTHCGIELDEDGSLDGNSDLTIRGRLLSLVEKVTYLKKKQAEKPVESDSKKSSTLQQLISETMVRWAQESVIEDPELVRAMFVLLHRQYDGIGGLVRALPKTYTIN

SEQ ID NO: 10 - DNA, 1374 bp, Artificial Sequence
  The sequence is synthetized.
aagttccactaccacaccctgagactgtacagcgccgtgtgcgccctgggcaaccacagagtggcccacgccctgtgcagccacgtggacgagccccagctgctgtacgccatcgagaacaagtacatgcccggcctgctgagagccggctactacgacctgctgatcgacatccacctgagcagctacgccaccgccagactgatgatgaacaacgagtacatcgtgcccatgaccgaggagaccaagagcatcaccctgttccccgacgagaacaagaagcacggcctgcccggcatcggcctgagcaccagcctgagacccagaatgcagttcagcagccccagcttcgtgagcatcagcaacgagtgctaccagtacagccccgagttccccctggacatcctgaagagcaagaccatccagatgctgaccgaggccgtgaaggagggcagcctgcacgccagagaccccgtgggcggcaccaccgagttcctgttcgtgcccctgatcaagctgttctacaccctgctgatcatgggcatcttccacaacgaggacctgaagcacatcctgcagctgatcgagcccagcgtgttcaaggaggccgccacccccgaggaggagagcgacaccctggagaaggagctgagcgtggacgacgccaagctgcagggcgccggcgaggaggaggccaagggcggcaagagacccaaggagggcctgctgcagatgaagctgcccgagcccgtgaagctgcagatgtgcctgctgctgcagtacctgtgcgactgccaggtgagacacagaatcgaggccatcgtggccttcagcgacgacttcgtggccaagctgcaggacaaccagagattcagatacaacgaggtgatgcaggccctgaacatgagcgccgccctgaccgccagaaagaccaaggagttcagaagccccccccaggagcagatcaacatgctgctgaacttcaaggacgacaagagcgagtgcccctgccccgaggagatcagagaccagctgctggacttccacgaggacctgatgacccactgcggcatcgagctggacgaggacggcagcctggacggcaacagcgacctgaccatcagaggcagactgctgagcctggtggagaaggtgacctacctgaagaagaagcaggccgagaagcccgtggagagcgacagcaagaagagcagcaccctgcagcagctgatcagcgagaccatggtgagatgggcccaggagagcgtgatcgaggaccccgagctggtgagagccatgttcgtgctgctgcacagacagtacgacggcatcggcggcctggtgagagccctgcccaagacctacaccatcaac

SEQ ID NO: 11 - protein, 569 aa, Artificial Sequence
  The sequence is synthetized.
GVSVEDTINLLASLGQIRSLLSVRMGKEEEKLMIRGLGDIMNNKVFYQHPNLMRALGMHETVMEVMVNVLGGGESKEITFPKMVANCCRFLCYFCRISRQNQKAMFDHLSYLLENSSVGLASPAMRGSTPLDVAAASVMDNNELALALREPDLEKVVRYLAGCGLQSCQMLVSKGYPDIGWNPVEGERYLDFLRFAVFCNGESVEENANVVVRLLIRRPECFGPALRGEGGNGLLAAMEEAIKIAEDPSRDGPSPNSGSSKTLDTEEEEDDTIHMGNAIMTFYSALIDLLGRCAPEMHLIHAGKGEAIRIRSILRSLIPLGDLVGVISIAFQMPTIAKDGNVVEPDMSAGFCPDHKAAMVLFLDRVYGIEVQDFLLHLLEVGFLPDLRAAASLDTAALSATDMALALNRYLCTAVLPLLTRCAPLFAGTEHHASLIDSLLHTVYRLSKGCSLTKAQRDSIEVCLLSICGQLRPSMMQHLLRRLVFDVPLLNEHAKMPLKLLTNHYERCWKYYCLPGGWGNFGAASEEELHLSRKLFWGIFDALSQKKYEQELFKLALPCLSAVAGALPP

SEQ ID NO: 12 - DNA, 1707 bp, Artificial Sequence
  The sequence is synthetized.
ggcgtgagcgtggaggacaccatcaacctgctggccagcctgggccagatcagaagcctgctgagcgtgagaatgggcaaggaggaggagaagctgatgatcagaggcctgggcgacatcatgaacaacaaggtgttctaccagcaccccaacctgatgagagccctgggcatgcacgagaccgtgatggaggtgatggtgaacgtgctgggcggcggcgagagcaaggagatcaccttccccaagatggtggccaactgctgcagattcctgtgctacttctgcagaatcagcagacagaaccagaaggccatgttcgaccacctgagctacctgctggagaacagcagcgtgggcctggccagccccgccatgagaggcagcacccccctggacgtggccgccgccagcgtgatggacaacaacgagctggccctggccctgagagagcccgacctggagaaggtggtgagatacctggccggctgcggcctgcagagctgccagatgctggtgagcaagggctaccccgacatcggctggaaccccgtggagggcgagagatacctggacttcctgagattcgccgtgttctgcaacggcgagagcgtggaggagaacgccaacgtggtggtgagactgctgatcagaagacccgagtgcttcggccccgccctgagaggcgagggcggcaacggcctgctggccgccatggaggaggccatcaagatcgccgaggaccccagcagagacggccccagccccaacagcggcagcagcaagaccctggacaccgaggaggaggaggacgacaccatccacatgggcaacgccatcatgaccttctacagcgccctgatcgacctgctgggcagatgcgcccccgagatgcacctgatccacgccggcaagggcgaggccatcagaatcagaagcatcctgagaagcctgatccccctgggcgacctggtgggcgtgatcagcatcgccttccagatgcccaccatcgccaaggacggcaacgtggtggagcccgacatgagcgccggcttctgccccgaccacaaggccgccatggtgctgttcctggacagagtgtacggcatcgaggtgcaggacttcctgctgcacctgctggaggtgggcttcctgcccgacctgagagccgccgccagcctggacaccgccgccctgagcgccaccgacatggccctggccctgaacagatacctgtgcaccgccgtgctgcccctgctgaccagatgcgcccccctgttcgccggcaccgagcaccacgccagcctgatcgacagcctgctgcacaccgtgtacagactgagcaagggctgcagcctgaccaaggcccagagagacagcatcgaggtgtgcctgctgagcatctgcggccagctgagacccagcatgatgcagcacctgctgagaagactggtgttcgacgtgcccctgctgaacgagcacgccaagatgcccctgaagctgctgaccaaccactacgagagatgctggaagtactactgcctgcccggcggctggggcaacttcggcgccgccagcgaggaggagctgcacctgagcagaaagctgttctggggcatcttcgacgccctgagccagaagaagtacgagcaggagctgttcaagctggccctgccctgcctgagcgccgtggccggcgccctgcccccc

SEQ ID NO: 13 - protein, 547 aa, Artificial Sequence
  The sequence is synthetized.
YFLSAASRPLCSGGHASNKEKEMVTSLFCKLGVLVRHRISLFGNDATSIVNCLHILGQTLDARTVMKTGLESVKSALRAFLDNAAEDLEKTMENLKQGQFTHTRNQPKGVTQIINYTTVALLPMLSSLFEHIGQHQFGEDLILEDVQVSCYRILTSLYALGTSKSIYVERQRSALGECLAAFAGAFPVAFLETHLDKHNIYSIYNTKSSRERAALSLPTNVEDVCPNIPSLEKLMEEIVELAESGIRYTQMPHVMEVILPMLCSYMSRWWEHGPENNPERAEMCCTALNSEHMNTLLGNILKIIYNNLGIDEGAWMKRLAVFSQPIINKVKPQLLKTHFLPLMEKLKKKAATVVSEEDHLKAEARGDMSEAELLILDEFTTLARDLYAFYPLLIRFVDYNRAKWLKEPNPEAEELFRMVAEVFIYWSKSHNFKREEQNFVVQNEINNMSFLITDTKSKMSKAAVSDQERKKMKRKGDRYSMQTSLIVAALKRLLPIGLNICAPGDQELIALAKNRFSLKDTEDEVRDIIRSNIHLQGKLEDPAIRWQ

SEQ ID NO: 14 - DNA, 1656 bp, Artificial Sequence
  The sequence is synthetized.
agatacagacacgactacttcctgagcgccgccagcagacccctgtgcagcggcggccacgccagcaacaaggagaaggagatggtgaccagcctgttctgcaagctgggcgtgctggtgagacacagaatcagcctgttcggcaacgacgccaccagcatcgtgaactgcctgcacatcctgggccagaccctggacgccagaaccgtgatgaagaccggcctggagagcgtgaagagcgccctgagagccttcctggacaacgccgccgaggacctggagaagaccatggagaacctgaagcagggccagttcacccacaccagaaaccagcccaagggcgtgacccagatcatcaactacaccaccgtggccctgctgcccatgctgagcagcctgttcgagcacatcggccagcaccagttcggcgaggacctgatcctggaggacgtgcaggtgagctgctacagaatcctgaccagcctgtacgccctgggcaccagcaagagcatctacgtggagagacagagaagcgccctgggcgagtgcctggccgccttcgccggcgccttccccgtggccttcctggagacccacctggacaagcacaacatctacagcatctacaacaccaagagcagcagagagagagccgccctgagcctgcccaccaacgtggaggacgtgtgccccaacatccccagcctggagaagctgatggaggagatcgtggagctggccgagagcggcatcagatacacccagatgccccacgtgatggaggtgatcctgcccatgctgtgcagctacatgagcagatggtgggagcacggccccgagaacaaccccgagagagccgagatgtgctgcaccgccctgaacagcgagcacatgaacaccctgctgggcaacatcctgaagatcatctacaacaacctgggcatcgacgagggcgcctggatgaagagactggccgtgttcagccagcccatcatcaacaaggtgaagccccagctgctgaagacccacttcctgcccctgatggagaagctgaagaagaaggccgccaccgtggtgagcgaggaggaccacctgaaggccgaggccagaggcgacatgagcgaggccgagctgctgatcctggacgagttcaccaccctggccagagacctgtacgccttctaccccctgctgatcagattcgtggactacaacagagccaagtggctgaaggagcccaaccccgaggccgaggagctgttcagaatggtggccgaggtgttcatctactggagcaagagccacaacttcaagagagaggagcagaacttcgtggtgcagaacgagatcaacaacatgagcttcctgatcaccgacaccaagagcaagatgagcaaggccgccgtgagcgaccaggagagaaagaagatgaagagaaagggcgacagatacagcatgcagaccagcctgatcgtggccgccctgaagagactgctgcccatcggcctgaacatctgcgcccccggcgaccaggagctgatcgccctggccaagaacagattcagcctgaaggacaccgaggacgaggtgagagacatcatcagaagcaacatccacctgcagggcaagctggaggaccccgccatcagatggcag

SEQ ID NO: 15 - protein, 385 aa, Artificial Sequence
  The sequence is synthetized.
YFEDKLIEDLAKPGAEPPEEDEGTKRVDPLHQLILLFSRTALTEKCKLEEDFLYMAYADIMAKSCHDEEDDDGEEEVKSFEEKEMEKQKLLYQQARLHDRGAAEMVLQTISASKGETGPMVAATLKLGIAILNGGNSTVQQKMLDYLKEKKDVGFFQSLAGLMQSCSVLDLNAFERQNKAEGLGMVTEEGSGEKVLQDDEFTCDLFRFLQLLCEGHNSDFQNYLRTQTGNNTTVNIIISTVDYLLRVQESISDFYWYYSGKDVIDEQGQRNFSKAIQVAKQVFNTLTEYIQGPCTGNQQSLAHSRLWDAVVGFLHVFAHMQMKLSQDSSQIELLKELMDLQKDMVVMLLSMLEGNVVNGTIGKQMVDMLVESSNNVEMILKFFDM

SEQ ID NO: 16 - DNA, 1155 bp, Artificial Sequence
  The sequence is synthetized.
tacttcgaggacaagctgatcgaggacctggccaagcccggcgccgagccccccgaggaggacgagggcaccaagagagtggaccccctgcaccagctgatcctgctgttcagcagaaccgccctgaccgagaagtgcaagctggaggaggacttcctgtacatggcctacgccgacatcatggccaagagctgccacgacgaggaggacgacgacggcgaggaggaggtgaagagcttcgaggagaaggagatggagaagcagaagctgctgtaccagcaggccagactgcacgacagaggcgccgccgagatggtgctgcagaccatcagcgccagcaagggcgagaccggccccatggtggccgccaccctgaagctgggcatcgccatcctgaacggcggcaacagcaccgtgcagcagaagatgctggactacctgaaggagaagaaggacgtgggcttcttccagagcctggccggcctgatgcagagctgcagcgtgctggacctgaacgccttcgagagacagaacaaggccgagggcctgggcatggtgaccgaggagggcagcggcgagaaggtgctgcaggacgacgagttcacctgcgacctgttcagattcctgcagctgctgtgcgagggccacaacagcgacttccagaactacctgagaacccagaccggcaacaacaccaccgtgaacatcatcatcagcaccgtggactacctgctgagagtgcaggagagcatcagcgacttctactggtactacagcggcaaggacgtgatcgacgagcagggccagagaaacttcagcaaggccatccaggtggccaagcaggtgttcaacaccctgaccgagtacatccagggcccctgcaccggcaaccagcagagcctggcccacagcagactgtgggacgccgtggtgggcttcctgcacgtgttcgcccacatgcagatgaagctgagccaggacagcagccagatcgagctgctgaaggagctgatggacctgcagaaggacatggtggtgatgctgctgagcatgctggagggcaacgtggtgaacggcaccatcggcaagcagatggtggacatgctggtggagagcagcaacaacgtggagatgatcctgaagttcttcgacatg

SEQ ID NO: 17 - protein, 61 aa, Artificial Sequence
  The sequence is synthetized.
LTSSDTFKEYDPDGKGVISKRDFHKAMESHKHYTQSETEFLLSCAETDENETLDYEEFVKR

SEQ ID NO: 18 - DNA, 183 bp, Artificial Sequence
  The sequence is synthetized.
ctgaccagcagcgacaccttcaaggagtacgaccccgacggcaagggcgtgatcagcaagagagacttccacaaggccatggagagccacaagcactacacccagagcgagaccgagttcctgctgagctgcgccgagaccgacgagaacgagaccctggactacgaggagttcgtgaagaga

SEQ ID NO: 19 - protein, 117 aa, Artificial Sequence
  The sequence is synthetized.
PAKDIGFNVAVLLTNLSEHMPNDTRLQTFLELAESVLNYFQPFLGRIEIMGSAKRIERVYFEISESSRTQWEKPQVKESKRQFIFDVVNEGGEKEKMELFVNFCEDTIFEMQLAAQI

SEQ ID NO: 20 - DNA, 351 bp, Artificial Sequence
  The sequence is synthetized.
cccgccaaggacatcggcttcaacgtggccgtgctgctgaccaacctgagcgagcacatgcccaacgacaccagactgcagaccttcctggagctggccgagagcgtgctgaactacttccagcccttcctgggcagaatcgagatcatgggcagcgccaagagaatcgagagagtgtacttcgagatcagcgagagcagcagaacccagtgggagaagccccaggtgaaggagagcaagagacagttcatcttcgacgtggtgaacgagggcggcgagaaggagaagatggagctgttcgtgaacttctgcgaggacaccatcttcgagatgcagctggccgcccagatc

SEQ ID NO: 21 - protein, 207 aa, Artificial Sequence
  The sequence is synthetized.
NFNPQPVDTSNITIPEKLEYFINKYAEHSHDKWSMDKLANGWIYGEIYSDSSKVQPLMKPYKLLSEKEKEIYRWPIKESLKTMLAWGWRIERTREGDSMALYNRTRRISQTSQVSVDAAHGYSPRAIDMSNVTLSRDLHAMAEMMAENYHNIWAKKKKMELESKGGGNHPLLVPYDTLTAKEKAKDREKAQDILKFLQINGYAVSRG

SEQ ID NO: 22 - DNA, 621 bp, Artificial Sequence
  The sequence is synthetized.
aacttcaacccccagcccgtggacaccagcaacatcaccatccccgagaagctggagtacttcatcaacaagtacgccgagcacagccacgacaagtggagcatggacaagctggccaacggctggatctacggcgagatctacagcgacagcagcaaggtgcagcccctgatgaagccctacaagctgctgagcgagaaggagaaggagatctacagatggcccatcaaggagagcctgaagaccatgctggcctggggctggagaatcgagagaaccagagagggcgacagcatggccctgtacaacagaaccagaagaatcagccagaccagccaggtgagcgtggacgccgcccacggctacagccccagagccatcgacatgagcaacgtgaccctgagcagagacctgcacgccatggccgagatgatggccgagaactaccacaacatctgggccaagaagaagaagatggagctggagagcaagggcggcggcaaccaccccctgctggtgccctacgacaccctgaccgccaaggagaaggccaaggacagagagaaggcccaggacatcctgaagttcctgcagatcaacggctacgccgtgagcagaggc

SEQ ID NO: 23 - protein, 156 aa, Artificial Sequence
  The sequence is synthetized.
QPVDTSNITIPEKLEYFINKYAEHSHDKWSMDKLANGWIYGEIYSDSSKVQPLMKPYKLLSEKEKEIYRWPIKESLKTMLAWGWRIERTREGDSMALYNRTRRISQTSQVSVDAAHGYSPRAIDMSNVTLSRDLHAMAEMMAENYHNIWAKKKKME

SEQ ID NO: 24 - DNA, 468 bp, Artificial Sequence
  The sequence is synthetized.
cagcccgtggacaccagcaacatcaccatccccgagaagctggagtacttcatcaacaagtacgccgagcacagccacgacaagtggagcatggacaagctggccaacggctggatctacggcgagatctacagcgacagcagcaaggtgcagcccctgatgaagccctacaagctgctgagcgagaaggagaaggagatctacagatggcccatcaaggagagcctgaagaccatgctggcctggggctggagaatcgagagaaccagagagggcgacagcatggccctgtacaacagaaccagaagaatcagccagaccagccaggtgagcgtggacgccgcccacggctacagccccagagccatcgacatgagcaacgtgaccctgagcagagacctgcacgccatggccgagatgatggccgagaactaccacaacatctgggccaagaagaagaagatggag

SEQ ID NO: 25 - protein, 69 aa, Artificial Sequence
  The sequence is synthetized.
IYRWPIKESLKTMLAWGWRIERTREGDSMALYNRTRRISQTSQVSVDAAHGYSPRAIDMSNVTLSRDLH

SEQ ID NO: 26 - DNA, 207 bp, Artificial Sequence
  The sequence is synthetized.
atctacagatggcccatcaaggagagcctgaagaccatgctggcctggggctggagaatcgagagaaccagagagggcgacagcatggccctgtacaacagaaccagaagaatcagccagaccagccaggtgagcgtggacgccgcccacggctacagccccagagccatcgacatgagcaacgtgaccctgagcagagacctgcac

SEQ ID NO: 27 - protein, 17 aa, Artificial Sequence
  The sequence is synthetized.
TRRISQTSQVSVDAAHG

SEQ ID NO: 28 - DNA, 51 bp, Artificial Sequence
  The sequence is synthetized.
accagaagaatcagccagaccagccaggtgagcgtggacgccgcccacggc

SEQ ID NO: 29 - protein, 206 aa, Artificial Sequence
  The sequence is synthetized.
NFNPQPVDTSNITIPEKLEYFINKYAEHSHDKWSMDKLANGWIYGEIYSDSSKIQPLMKPYKLLSEKEKEIYRWPIKESLKTMLAWGWRIERTREGDSMALYNRTRRISQTSQVSIDAAHGYSPRAIDMSNVTLSRDLHAMAEMMAENYHNIWAKKKKLELESKGGGNHPLLVPYDTLTAKEKAKDREKAQDILKFLQINGYAVSR

SEQ ID NO: 30 - DNA, 618 bp, Artificial Sequence
  The sequence is synthetized.
aacttcaacccccagcccgtggacaccagcaacatcaccatccccgagaagctggagtacttcatcaacaagtacgccgagcacagccacgacaagtggagcatggacaagctggccaacggctggatctacggcgagatctacagcgacagcagcaagatccagcccctgatgaagccctacaagctgctgagcgagaaggagaaggagatctacagatggcccatcaaggagagcctgaagaccatgctggcctggggctggagaatcgagagaaccagagagggcgacagcatggccctgtacaacagaaccagaagaatcagccagaccagccaggtgagcatcgacgccgcccacggctacagccccagagccatcgacatgagcaacgtgaccctgagcagagacctgcacgccatggccgagatgatggccgagaactaccacaacatctgggccaagaagaagaagctggagctggagagcaagggcggcggcaaccaccccctgctggtgccctacgacaccctgaccgccaaggagaaggccaaggacagagagaaggcccaggacatcctgaagttcctgcagatcaacggctacgccgtgagcaga